European Patent Specification EP 3 393 495 B1, published December 6, 2023. Title: Small Molecule Inhibitors of HLA-DR3 Binding for Treating Autoimmune Thyroiditis. Applicant: Tomer, Yaron Osman, Roman. The sequence listing filed with the application follows.

SEQUENCE LISTING (5 sequences)

SEQ ID NO: 1 - protein, 19 aa, Homo sapiens
IPDNLFLKSDGRIKYTLNK

SEQ ID NO: 2 - protein, 15 aa, Artificial Sequence
  synthetic peptide
LSSVVVDPSIRHFDV

SEQ ID NO: 3 - protein, 15 aa, Artificial Sequence
  synthetic peptide
HDLFSRIDSSVVVVP

SEQ ID NO: 4 - DNA, 15 bp, Artificial Sequence
  synthetic oligonucleotide
cgcttcgacagcgac

SEQ ID NO: 5 - DNA, 18 bp, Artificial Sequence
  synthetic oligonucleotide
gacaaatccacactccac